European Patent Application EP 4 365 198 A1, published May 8, 2024. Title: ANTI-CD3 ANTIBODY AND USE THEREOF. Applicant: AMPSOURCE BIOPHARMA SHANGHAI INC. Application EP22831732.7. The sequence listing filed with the application follows.

SEQUENCE LISTING (119 sequences)

SEQ ID NO: 1 - protein, 119 aa, Artificial sequence
  AP191 heavy chain variable region
QVQLQQSGPELVKPGASMKMSCKASGYTFTSYYIHWVKQRPGQGLEWIGWIYPGDGSTKFNEKFRGKTSLTADKSSNTAYMFLSSLTSEDSAIYFCARDGYSLYYFEFWGHGTTLTVSS

SEQ ID NO: 2 - protein, 112 aa, Artificial sequence
  AP191 light chain variable region
DIVMSQSPSSLAVSAGETVTMSCKSSQSLLNSRTRKTYLAWYQQKPGQSPKLLIYWASTRDSGVPDRFTGSGSGTDFTLTISSVQAEDLAVYYCVQSYTLRTFGGGTKLEIK

SEQ ID NO: 3 - protein, 125 aa, Artificial sequence
  AP591 heavy chain variable region
EVQLVESGGGLVQPKGSLKLSCAASGFTFNTYAMNWVRQAPGKGLEWVGRIRSKINNYATYYADSVRDRFTISRDDSQSMLYLQMSNLKTEDTAMYYCVRHDNFYGSTYSWFADWGQGTLVTVSA

SEQ ID NO: 4 - protein, 108 aa, Artificial sequence
  AP591 light chain variable region
AVVTQESALTTSPGETVTLTCRSSTGVVTTSNYANWVQEKPDHLFTGLIGATNYRVPGVPARFSGSLIGDKAALTITGAQTEDEAIYFCVLWYSNHWVFGGGTKLTVL

SEQ ID NO: 5 - protein, 117 aa, Artificial sequence
  AP831 heavy chain variable region
QVQLQQSGPELVKPGTSVKMSCKASGYTFTNNYIHWVKEKPGEGLEWIGWIYPGDGTTKYNEKFKGKTTLASDKSSNTVYMFLSSLTSEDSAIYFCTRNNNYYFDYWGQGTTLTVSS

SEQ ID NO: 6 - protein, 112 aa, Artificial sequence
  AP831 light chain variable region
DIVMSQSPSSLAVSAGEKVTMNCKSSQSLFNSRTRKNYLAWYQQKPGQSPKLLIYWASTRESGVPDRFTGSGSGTDFTLTISSVQAEDLALYYCKQSFILRTFGGGTKLEIK

SEQ ID NO: 7 - protein, 5 aa, Artificial sequence
  Kabat AP191 CDR-H1
SYYIH

SEQ ID NO: 8 - protein, 17 aa, Artificial sequence
  Kabat AP191 CDR-H2
WIYPGDGSTKFNEKFRG

SEQ ID NO: 9 - protein, 10 aa, Artificial sequence
  Kabat AP191 CDR-H3
DGYSLYYFEF

SEQ ID NO: 10 - protein, 17 aa, Artificial sequence
  Kabat AP191 CDR-L1
KSSQSLLNSRTRKTYLA

SEQ ID NO: 11 - protein, 7 aa, Artificial sequence
  Kabat AP191 CDR-L2
WASTRDS

SEQ ID NO: 12 - protein, 8 aa, Artificial sequence
  Kabat/IMGT AP191 CDR-L3
VQSYTLRT

SEQ ID NO: 13 - protein, 8 aa, Artificial sequence
  IMGT AP191 CDR-H1
GYTFTSYY

SEQ ID NO: 14 - protein, 8 aa, Artificial sequence
  IMGT AP191 CDR-H2
IYPGDGST

SEQ ID NO: 15 - protein, 12 aa, Artificial sequence
  IMGT AP191 CDR-H3
ARDGYSLYYFEF

SEQ ID NO: 16 - protein, 12 aa, Artificial sequence
  IMGT AP191 CDR-L1
QSLLNSRTRKTY

SEQ ID NO: 17 - protein, 3 aa, Artificial sequence
  IMGT AP191 CDR-L2
WAS

SEQ ID NO: 18 - protein, 5 aa, Artificial sequence
  Kabat AP591 CDR-H1
TYAMN

SEQ ID NO: 19 - protein, 19 aa, Artificial sequence
  Kabat AP591 CDR-H2
RIRSKINNYATYYADSVRD

SEQ ID NO: 20 - protein, 14 aa, Artificial sequence
  Kabat AP591 CDR-H3
HDNFYGSTYSWFAD

SEQ ID NO: 21 - protein, 14 aa, Artificial sequence
  Kabat AP591 CDR-L1
RSSTGVVTTSNYAN

SEQ ID NO: 22 - protein, 7 aa, Artificial sequence
  Kabat AP591 CDR-L2
ATNYRVP

SEQ ID NO: 23 - protein, 9 aa, Artificial sequence
  Kabat/IMGT AP591 CDR-L3
VLWYSNHWV

SEQ ID NO: 24 - protein, 8 aa, Artificial sequence
  IMGT AP591 CDR-H1
GFTFNTYA

SEQ ID NO: 25 - protein, 10 aa, Artificial sequence
  IMGT AP591 CDR-H2
IRSKINNYAT

SEQ ID NO: 26 - protein, 16 aa, Artificial sequence
  IMGT AP591 CDR-H3
VRHDNFYGSTYSWFAD

SEQ ID NO: 27 - protein, 9 aa, Artificial sequence
  IMGT AP591 CDR-L1
TGVVTTSNY

SEQ ID NO: 28 - protein, 3 aa, Artificial sequence
  IMGT AP591 CDR-L2
ATN

SEQ ID NO: 29 - protein, 5 aa, Artificial sequence
  Kabat AP831 CDR-H1
NNYIH

SEQ ID NO: 30 - protein, 17 aa, Artificial sequence
  Kabat AP831 CDR-H2
WIYPGDGTTKYNEKFKG

SEQ ID NO: 31 - protein, 8 aa, Artificial sequence
  Kabat AP831 CDR-H3
NNNYYFDY

SEQ ID NO: 32 - protein, 17 aa, Artificial sequence
  Kabat AP831 CDR-L1
KSSQSLFNSRTRKNYLA

SEQ ID NO: 33 - protein, 7 aa, Artificial sequence
  Kabat AP831 CDR-L2
WASTRES

SEQ ID NO: 34 - protein, 8 aa, Artificial sequence
  Kabat/IMGT AP831 CDR-L3
KQSFILRT

SEQ ID NO: 35 - protein, 8 aa, Artificial sequence
  IMGT AP831 CDR-H1
GYTFTNNY

SEQ ID NO: 36 - protein, 8 aa, Artificial sequence
  IMGT AP831 CDR-H2
IYPGDGTT

SEQ ID NO: 37 - protein, 10 aa, Artificial sequence
  IMGT AP831 CDR-H3
TRNNNYYFDY

SEQ ID NO: 38 - protein, 12 aa, Artificial sequence
  IMGT AP831 CDR-L1
QSLFNSRTRKNY

SEQ ID NO: 39 - protein, 3 aa, Artificial sequence
  IMGT AP831 CDR-L2
WAS

SEQ ID NO: 40 - protein, 117 aa, Artificial sequence
  AB610 heavy chain variable region
EVQLLESGGGLVQPGGSLKLSCAASGYTFTNNYIHWVRQAPGKGLEWIGWIYPGDGTTKYNEKFKGKTTLASDDSKNTAYLQMNNLKTEDTAMYFCTRNNNYYFDYWGQGTLVTVSS

SEQ ID NO: 41 - protein, 111 aa, Artificial sequence
  AB610 light chain variable region
EIVVTQEPSLTVSPGGTVTLTCRSSQSLFNSRTRKNYLAWVQEKPGQAPRGLIYWASTRESGTPARFSGSLLGGKAALTLSGVQPEDEAIYYCKQSFILRTFGGGTKLEIK

SEQ ID NO: 42 - protein, 117 aa, Artificial sequence
  AB611 heavy chain variable region
EVQLVQSGAEVKKPGSSVKVSCKASGYTFTNNYIHWVKEKPGQGLEWIGWIYPGDGTTKYNEKFKGKTTLASDKSTNTAYMELSSLRSEDTAIYFCTRNNNYYFDYWGQGTTVTVSS

SEQ ID NO: 43 - protein, 112 aa, Artificial sequence
  AB611 light chain variable region
DIVMTQSPDSLAVSLGERATMNCKSSQSLFNSRTRKNYLAWYQQKPGESPKLLIYWASTRESGVPDRFSGSGSGTDFTLTISSLQAEDVAVYYCKQSFILRTFGGGTKVEIK

SEQ ID NO: 44 - protein, 119 aa, Artificial sequence
  AB612 heavy chain variable region
EVQLLESGGGLVQPGGSLKLSCAASGYTFTSYYIHWVRQAPGKGLEWVGWIYPGEGSTKFNEKFRGRFTISRDDSKNTAYLQMNNLKTEDTAMYFCAREGYSLYYFEFWGQGTLVTVSS

SEQ ID NO: 45 - protein, 111 aa, Artificial sequence
  AB612 light chain variable region
EIVVTQEPSLTVSPGGTVTLTCRSSQSLLNSRTRKTYLAWVQEKPDHLFTGLIYWASTRDPGTPARFSGSLLGGKAALTLSGVQPEDEAIYYCVQSYTLRTFGGGTKLEIK

SEQ ID NO: 46 - protein, 119 aa, Artificial sequence
  AB613 heavy chain variable region
EVQLVQSGAEVKKPGSSVKVSCKASGYTFTSYYIHWVRQAPGQGLEWMGWIYPGEGSTKFNEKFRGRTTLTADKSTNTAYMELSSLRSEDTAVYFCAREGYSLYYFEFWGQGTTVTVSS

SEQ ID NO: 47 - protein, 112 aa, Artificial sequence
  AB613 light chain variable region
DIVMTQSPDSLAVSLGERATINCKSSQSLLNSRTRKTYLAWYQQKPGESPKLLIYWASTRDSGVPDRFSGSGSGTDFTLTISSLQAEDVAVYYCVQSYTLRTFGGGTKVEIK

SEQ ID NO: 48 - protein, 125 aa, Artificial sequence
  AB614 heavy chain variable region
EVQLLESGGGLVQPGGSLKLSCAASGFTFNTYAMNWVRQAPGKGLEWVGRIRSKINNYATYYADSVKDRFTISRDDSKNTAYLQMNNLKTEDTAMYYCVRHDNFYGSTYSWFADWGQGTLVTVSS

SEQ ID NO: 49 - protein, 109 aa, Artificial sequence
  AB614 light chain variable region
ELVVTQEPSLTVSPGGTVTLTCRSSTGVVTTSNYANWVQEKPDHLFTGLIGATNYRAPGTPARFSGSLLGGKAALTLSGVQPEDEAIYFCVLWYSNHWVFGGGTKLTVL

SEQ ID NO: 50 - protein, 17 aa, Artificial sequence
  Kabat AB610 CDR-L1
RSSQSLFNSRTRKNYLA

SEQ ID NO: 51 - protein, 17 aa, Artificial sequence
  Kabat AB612 CDR-H2
WIYPGEGSTKFNEKFRG

SEQ ID NO: 52 - protein, 10 aa, Artificial sequence
  Kabat AB612 CDR-H3
EGYSLYYFEF

SEQ ID NO: 53 - protein, 17 aa, Artificial sequence
  Kabat AB612 CDR-L1
RSSQSLLNSRTRKTYLA

SEQ ID NO: 54 - protein, 7 aa, Artificial sequence
  Kabat AB612 CDR-L2
WASTRDP

SEQ ID NO: 55 - protein, 8 aa, Artificial sequence
  IMGT AB612 CDR-H2
IYPGEGST

SEQ ID NO: 56 - protein, 12 aa, Artificial sequence
  IMGT AB612 CDR-H3
AREGYSLYYFEF

SEQ ID NO: 57 - protein, 19 aa, Artificial sequence
  Kabat AB614 CDR-H2
RIRSKINNYATYYADSVKD

SEQ ID NO: 58 - protein, 7 aa, Artificial sequence
  Kabat AB614 CDR-L2
ATNYRAP

SEQ ID NO: 59 - protein, 107 aa, Artificial sequence [sequence omitted]

SEQ ID NO: 60 - protein, 330 aa, Artificial sequence
  amino acid sequence of wild-type IgG1
ASTKGPSVFPLAPSSKSTSGGTAALGCLVKDYFPEPVTVSWNSGALTSGVHTFPAVLQSSGLYSLSSVVTVPSSSLGTQTYICNVNHKPSNTKVDKRVEPKSCDKTHTCPPCPAPELLGGPSVFLFPPKPKDTLMISRTPEVTCVVVDVSHEDPEVKFNWYVDGVEVHNAKTKPREEQYNSTYRVVSVLTVLHQDWLNGKEYKCKVSNKALPAPIEKTISKAKGQPREPQVYTLPPSREEMTKNQVSLTCLVKGFYPSDIAVEWESNGQPENNYKTTPPVLDSDGSFFLYSKLTVDKSRWQQGNVFSCSVMHEALHNHYTQKSLSLSPGK

SEQ ID NO: 61 - protein, 330 aa, Artificial sequence
  amino acid sequence of the constant region of IgG1(N297A) mutant
ASTKGPSVFPLAPSSKSTSGGTAALGCLVKDYFPEPVTVSWNSGALTSGVHTFPAVLQSSGLYSLSSVVTVPSSSLGTQTYICNVNHKPSNTKVDKRVEPKSCDKTHTCPPCPAPELLGGPSVFLFPPKPKDTLMISRTPEVTCVVVDVSHEDPEVKFNWYVDGVEVHNAKTKPREEQYASTYRVVSVLTVLHQDWLNGKEYKCKVSNKALPAPIEKTISKAKGQPREPQVYTLPPSREEMTKNQVSLTCLVKGFYPSDIAVEWESNGQPENNYKTTPPVLDSDGSFFLYSKLTVDKSRWQQGNVFSCSVMHEALHNHYTQKSLSLSPGK

SEQ ID NO: 62 - protein, 330 aa, Artificial sequence
  amino acid sequence of the constant region of IgG1(L234A, L235A) mutant
ASTKGPSVFPLAPSSKSTSGGTAALGCLVKDYFPEPVTVSWNSGALTSGVHTFPAVLQSSGLYSLSSVVTVPSSSLGTQTYICNVNHKPSNTKVDKRVEPKSCDKTHTCPPCPAPEAAGGPSVFLFPPKPKDTLMISRTPEVTCVVVDVSHEDPEVKFNWYVDGVEVHNAKTKPREEQYNSTYRVVSVLTVLHQDWLNGKEYKCKVSNKALPAPIEKTISKAKGQPREPQVYTLPPSREEMTKNQVSLTCLVKGFYPSDIAVEWESNGQPENNYKTTPPVLDSDGSFFLYSKLTVDKSRWQQGNVFSCSVMHEALHNHYTQKSLSLSPGK

SEQ ID NO: 63 - protein, 327 aa, Artificial sequence
  amino acid sequence of wild-type IgG4
ASTKGPSVFPLAPCSRSTSESTAALGCLVKDYFPEPVTVSWNSGALTSGVHTFPAVLQSSGLYSLSSVVTVPSSSLGTKTYTCNVDHKPSNTKVDKRVESKYGPPCPSCPAPEFLGGPSVFLFPPKPKDTLMISRTPEVTCVVVDVSQEDPEVQFNWYVDGVEVHNAKTKPREEQFNSTYRVVSVLTVLHQDWLNGKEYKCKVSNKGLPSSIEKTISKAKGQPREPQVYTLPPSQEEMTKNQVSLTCLVKGFYPSDIAVEWESNGQPENNYKTTPPVLDSDGSFFLYSRLTVDKSRWQEGNVFSCSVMHEALHNHYTQKSLSLSLGK

SEQ ID NO: 64 - protein, 327 aa, Artificial sequence
  amino acid sequence of the constant region of IgG4(S228P) mutant
ASTKGPSVFPLAPCSRSTSESTAALGCLVKDYFPEPVTVSWNSGALTSGVHTFPAVLQSSGLYSLSSVVTVPSSSLGTKTYTCNVDHKPSNTKVDKRVESKYGPPCPPCPAPEFLGGPSVFLFPPKPKDTLMISRTPEVTCVVVDVSQEDPEVQFNWYVDGVEVHNAKTKPREEQFNSTYRVVSVLTVLHQDWLNGKEYKCKVSNKGLPSSIEKTISKAKGQPREPQVYTLPPSQEEMTKNQVSLTCLVKGFYPSDIAVEWESNGQPENNYKTTPPVLDSDGSFFLYSRLTVDKSRWQEGNVFSCSVMHEALHNHYTQKSLSLSLGK

SEQ ID NO: 65 - protein, 444 aa, Artificial sequence
  AB610 heavy chain amino acid sequence
EVQLLESGGGLVQPGGSLKLSCAASGYTFTNNYIHWVRQAPGKGLEWIGWIYPGDGTTKYNEKFKGKTTLASDDSKNTAYLQMNNLKTEDTAMYFCTRNNNYYFDYWGQGTLVTVSSASTKGPSVFPLAPCSRSTSESTAALGCLVKDYFPEPVTVSWNSGALTSGVHTFPAVLQSSGLYSLSSVVTVPSSSLGTKTYTCNVDHKPSNTKVDKRVESKYGPPCPPCPAPEFLGGPSVFLFPPKPKDTLMISRTPEVTCVVVDVSQEDPEVQFNWYVDGVEVHNAKTKPREEQFNSTYRVVSVLTVLHQDWLNGKEYKCKVSNKGLPSSIEKTISKAKGQPREPQVYTLPPSQEEMTKNQVSLTCLVKGFYPSDIAVEWESNGQPENNYKTTPPVLDSDGSFFLYSRLTVDKSRWQEGNVFSCSVMHEALHNHYTQKSLSLSLGK

SEQ ID NO: 66 - protein, 218 aa, Artificial sequence
  AB610 light chain amino acid sequence
EIVVTQEPSLTVSPGGTVTLTCRSSQSLFNSRTRKNYLAWVQEKPGQAPRGLIYWASTRESGTPARFSGSLLGGKAALTLSGVQPEDEAIYYCKQSFILRTFGGGTKLEIKRTVAAPSVFIFPPSDEQLKSGTASVVCLLNNFYPREAKVQWKVDNALQSGNSQESVTEQDSKDSTYSLSSTLTLSKADYEKHKVYACEVTHQGLSSPVTKSFNRGEC

SEQ ID NO: 67 - DNA, 1332 bp, Artificial sequence
  AB610 heavy chain nucleotide sequence
gaggtgcagctgctggagtctggaggaggactggtgcagcctggaggaagcctgaagctgtcttgcgccgcttccggctacaccttcacaaacaattatatccattgggtgaggcaggctccaggcaagggactggagtggatcggctggatctaccctggcgatggcaccacaaagtataacgagaagtttaagggcaagaccacactggcctctgacgattccaagaataccgcttacctgcagatgaacaatctgaagaccgaggatacagctatgtacttctgcacccggaacaataactactattttgactattggggccagggcaccctggtgacagtgtccagcgcctctaccaagggcccttccgtgttccctctggccccatgttcccgcagcacctctgagtccacagccgctctgggctgcctggtgaaggactatttccccgagcctgtgaccgtgtcctggaacagcggcgctctgacctccggagtgcacacatttcccgccgtgctgcagtcttccggcctgtacagcctgagctctgtggtgaccgtgccatccagctctctgggcaccaagacatatacctgtaacgtggatcataagccctccaatacaaaggtggacaagcgcgtggagagcaagtacggaccaccatgtcctccatgcccagctcccgagtttctgggcggccctagcgtgttcctgtttccccctaagccaaaggataccctgatgatcagcaggacccctgaggtgacatgcgtggtggtggacgtgtcccaggaggacccagaggtgcagttcaactggtacgtggacggcgtggaggtgcacaatgccaagaccaagcctcgggaggagcagtttaattccacctacagagtggtgagcgtgctgacagtgctgcatcaggactggctgaacggcaaggagtataagtgtaaggtgtccaataagggcctgccatccagcatcgagaagaccatcagcaaggctaagggccagcccagggagcctcaggtgtacacactgccaccctctcaggaggagatgaccaagaaccaggtgtccctgacatgcctggtgaagggcttctatccttccgatatcgccgtggagtgggagagcaatggccagccagagaacaattacaagaccacacctccagtgctggattctgacggctccttctttctgtattcccggctgaccgtggacaagagcagatggcaggagggcaacgtgtttagctgttctgtgatgcatgaggctctgcacaatcattacacacagaagtccctgagcctgtctctgggcaag

SEQ ID NO: 68 - DNA, 654 bp, Artificial sequence
  AB610 light chain nucleotide sequence
gagatcgtggtgacccaggagccaagcctgacagtgtctcccggcggcaccgtgacactgacctgtagatcttcccagtccctgttcaacagcaggacccggaagaattacctggcctgggtgcaggagaagccaggacaggctccaaggggactgatctattgggcttctaccagggagtccggcacaccagctcggtttagcggatctctgctgggaggcaaggctgccctgaccctgtccggagtgcagcccgaggacgaggctatctactattgcaagcagagcttcatcctgaggacctttggcggcggcacaaagctggagatcaagaggaccgtggctgccccctccgtgttcatctttcccccttccgatgagcagctgaagtccggcacagccagcgtggtgtgcctgctgaacaatttctaccctagagaggctaaggtgcagtggaaggtggacaacgccctgcagagcggcaattctcaggagtccgtgaccgagcaggatagcaaggactctacatattccctgtccagcacactgaccctgagcaaggctgattacgagaagcacaaggtgtatgcctgtgaggtgacccatcagggcctgtcttcccctgtgacaaagtctttcaaccggggcgagtgc

SEQ ID NO: 69 - protein, 444 aa, Artificial sequence
  AB611 heavy chain amino acid sequence
EVQLVQSGAEVKKPGSSVKVSCKASGYTFTNNYIHWVKEKPGQGLEWIGWIYPGDGTTKYNEKFKGKTTLASDKSTNTAYMELSSLRSEDTAIYFCTRNNNYYFDYWGQGTTVTVSSASTKGPSVFPLAPCSRSTSESTAALGCLVKDYFPEPVTVSWNSGALTSGVHTFPAVLQSSGLYSLSSVVTVPSSSLGTKTYTCNVDHKPSNTKVDKRVESKYGPPCPPCPAPEFLGGPSVFLFPPKPKDTLMISRTPEVTCVVVDVSQEDPEVQFNWYVDGVEVHNAKTKPREEQFNSTYRVVSVLTVLHQDWLNGKEYKCKVSNKGLPSSIEKTISKAKGQPREPQVYTLPPSQEEMTKNQVSLTCLVKGFYPSDIAVEWESNGQPENNYKTTPPVLDSDGSFFLYSRLTVDKSRWQEGNVFSCSVMHEALHNHYTQKSLSLSLGK

SEQ ID NO: 70 - protein, 219 aa, Artificial sequence
  AB611 light chain amino acid sequence
DIVMTQSPDSLAVSLGERATMNCKSSQSLFNSRTRKNYLAWYQQKPGESPKLLIYWASTRESGVPDRFSGSGSGTDFTLTISSLQAEDVAVYYCKQSFILRTFGGGTKVEIKRTVAAPSVFIFPPSDEQLKSGTASVVCLLNNFYPREAKVQWKVDNALQSGNSQESVTEQDSKDSTYSLSSTLTLSKADYEKHKVYACEVTHQGLSSPVTKSFNRGEC

SEQ ID NO: 71 - DNA, 1332 bp, Artificial sequence
  AB611 heavy chain nucleotide sequence
gaggtgcagctggtgcagagcggagctgaggtgaagaagccaggcagctctgtgaaggtgagctgtaaggcttctggctacacattcaccaataactatatccactgggtgaaagaaaagccaggacagggcctggaatggatcggatggatctaccccggcgatggtactaccaaatacaatgaaaagtttaagggcaagaccacactggcgagcgacaagtctacaaataccgcttacatggagctgtccagcctgaggtctgaggataccgccatctacttctgcacacggaacaacaactactacttcgactactggggccagggcaccacagtgaccgtgtcttccgcctctaccaagggcccttccgtgttccctctggccccatgttcccgcagcacctctgagtccacagccgctctgggctgcctggtgaaggactatttccccgagcctgtgaccgtgtcctggaacagcggcgctctgacctccggagtgcacacatttcccgccgtgctgcagtcttccggcctgtacagcctgagctctgtggtgaccgtgccatccagctctctgggcaccaagacatatacctgtaacgtggatcataagccctccaatacaaaggtggacaagcgcgtggagagcaagtacggaccaccatgtcctccatgcccagctcccgagtttctgggcggccctagcgtgttcctgtttccccctaagccaaaggataccctgatgatcagcaggacccctgaggtgacatgcgtggtggtggacgtgtcccaggaggacccagaggtgcagttcaactggtacgtggacggcgtggaggtgcacaatgccaagaccaagcctcgggaggagcagtttaattccacctacagagtggtgagcgtgctgacagtgctgcatcaggactggctgaacggcaaggagtataagtgtaaggtgtccaataagggcctgccatccagcatcgagaagaccatcagcaaggctaagggccagcccagggagcctcaggtgtacacactgccaccctctcaggaggagatgaccaagaaccaggtgtccctgacatgcctggtgaagggcttctatccttccgatatcgccgtggagtgggagagcaatggccagccagagaacaattacaagaccacacctccagtgctggattctgacggctccttctttctgtattcccggctgaccgtggacaagagcagatggcaggagggcaacgtgtttagctgttctgtgatgcatgaggctctgcacaatcattacacacagaagtccctgagcctgtctctgggcaag

SEQ ID NO: 72 - DNA, 657 bp, Artificial sequence
  AB611 light chain nucleotide sequence
gatatcgtgatgacacagtccccagacagcctggccgtgagcctgggagagcgggctaccatgaactgtaagagctctcagtctctgttcaactctagaacacgcaaaaactacctggcctggtatcagcagaagcctggcgagtctccaaagctgctgatctactgggcttctaccagagagtccggagtgcctgatcgcttctccggaagcggctctggcacagactttacactgaccatctccagcctgcaggccgaggatgtggccgtgtactactgtaaacaaagcttcatcctgaggacctttggcggaggcacaaaggtggagatcaagaggaccgtggctgccccctccgtgttcatctttcccccttccgatgagcagctgaagtccggcacagccagcgtggtgtgcctgctgaacaatttctaccctagagaggctaaggtgcagtggaaggtggacaacgccctgcagagcggcaattctcaggagtccgtgaccgagcaggatagcaaggactctacatattccctgtccagcacactgaccctgagcaaggctgattacgagaagcacaaggtgtatgcctgtgaggtgacccatcagggcctgtcttcccctgtgacaaagtctttcaaccggggcgagtgc

SEQ ID NO: 73 - protein, 446 aa, Artificial sequence
  AB612 heavy chain amino acid sequence
EVQLLESGGGLVQPGGSLKLSCAASGYTFTSYYIHWVRQAPGKGLEWVGWIYPGEGSTKFNEKFRGRFTISRDDSKNTAYLQMNNLKTEDTAMYFCAREGYSLYYFEFWGQGTLVTVSSASTKGPSVFPLAPCSRSTSESTAALGCLVKDYFPEPVTVSWNSGALTSGVHTFPAVLQSSGLYSLSSVVTVPSSSLGTKTYTCNVDHKPSNTKVDKRVESKYGPPCPPCPAPEFLGGPSVFLFPPKPKDTLMISRTPEVTCVVVDVSQEDPEVQFNWYVDGVEVHNAKTKPREEQFNSTYRVVSVLTVLHQDWLNGKEYKCKVSNKGLPSSIEKTISKAKGQPREPQVYTLPPSQEEMTKNQVSLTCLVKGFYPSDIAVEWESNGQPENNYKTTPPVLDSDGSFFLYSRLTVDKSRWQEGNVFSCSVMHEALHNHYTQKSLSLSLGK

SEQ ID NO: 74 - protein, 218 aa, Artificial sequence
  AB612 light chain amino acid sequence
EIVVTQEPSLTVSPGGTVTLTCRSSQSLLNSRTRKTYLAWVQEKPDHLFTGLIYWASTRDPGTPARFSGSLLGGKAALTLSGVQPEDEAIYYCVQSYTLRTFGGGTKLEIKRTVAAPSVFIFPPSDEQLKSGTASVVCLLNNFYPREAKVQWKVDNALQSGNSQESVTEQDSKDSTYSLSSTLTLSKADYEKHKVYACEVTHQGLSSPVTKSFNRGEC

SEQ ID NO: 75 - DNA, 1338 bp, Artificial sequence
  AB612 heavy chain nucleotide sequence
gaagtccagctgctggagagcggcggcggactggtgcagccaggcggcagcctgaagctgtcttgtgccgcttccggctacacattcacctcttactatatccattgggtgcggcaggctcctggcaagggcctggaatgggtgggctggatctatccaggcgagggctccaccaagtttaacgagaagttcaggggccggtttaccatcagcagggacgattctaagaatacagcctacctgcagatgaataatctgaagaccgaggacacagccatgtacttttgcgctcgggagggctatagcctgtactattttgagttctggggtcagggcaccctggtcacagtgtcttccgcctctaccaagggcccttccgtgttccctctggccccatgttcccgcagcacctctgagtccacagccgctctgggctgcctggtgaaggactatttccccgagcctgtgaccgtgtcctggaacagcggcgctctgacctccggagtgcacacatttcccgccgtgctgcagtcttccggcctgtacagcctgagctctgtggtgaccgtgccatccagctctctgggcaccaagacatatacctgtaacgtggatcataagccctccaatacaaaggtggacaagcgcgtggagagcaagtacggaccaccatgtcctccatgcccagctcccgagtttctgggcggccctagcgtgttcctgtttccccctaagccaaaggataccctgatgatcagcaggacccctgaggtgacatgcgtggtggtggacgtgtcccaggaggacccagaggtgcagttcaactggtacgtggacggcgtggaggtgcacaatgccaagaccaagcctcgggaggagcagtttaattccacctacagagtggtgagcgtgctgacagtgctgcatcaggactggctgaacggcaaggagtataagtgtaaggtgtccaataagggcctgccatccagcatcgagaagaccatcagcaaggctaagggccagcccagggagcctcaggtgtacacactgccaccctctcaggaggagatgaccaagaaccaggtgtccctgacatgcctggtgaagggcttctatccttccgatatcgccgtggagtgggagagcaatggccagccagagaacaattacaagaccacacctccagtgctggattctgacggctccttctttctgtattcccggctgaccgtggacaagagcagatggcaggagggcaacgtgtttagctgttctgtgatgcatgaggctctgcacaatcattacacacagaagtccctgagcctgtctctgggcaag

SEQ ID NO: 76 - DNA, 654 bp, Artificial sequence
  AB612 light chain nucleotide sequence
gaaattgtggtgacccaggagccttccctgacagtgagcccaggcggcacagtgaccctgacatgtagaagctctcagtctctgctgaactccagaacccgcaagacatacctggcttgggtccaggagaagcctgatcatctgttcaccggcctgatctattgggcttccaccagggacccaggaacacctgctcggttttccggaagcctgctgggaggcaaggccgctctgaccctgtctggagtgcagccagaagatgaagccatctactattgcgtgcagtcctacaccctgagaacattcggcggcggcaccaagctggagatcaagaggaccgtggctgccccctccgtgttcatctttcccccttccgatgagcagctgaagtccggcacagccagcgtggtgtgcctgctgaacaatttctaccctagagaggctaaggtgcagtggaaggtggacaacgccctgcagagcggcaattctcaggagtccgtgaccgagcaggatagcaaggactctacatattccctgtccagcacactgaccctgagcaaggctgattacgagaagcacaaggtgtatgcctgtgaggtgacccatcagggcctgtcttcccctgtgacaaagtctttcaaccggggcgagtgc

SEQ ID NO: 77 - protein, 446 aa, Artificial sequence
  AB613 heavy chain amino acid sequence
EVQLVQSGAEVKKPGSSVKVSCKASGYTFTSYYIHWVRQAPGQGLEWMGWIYPGEGSTKFNEKFRGRTTLTADKSTNTAYMELSSLRSEDTAVYFCAREGYSLYYFEFWGQGTTVTVSSASTKGPSVFPLAPCSRSTSESTAALGCLVKDYFPEPVTVSWNSGALTSGVHTFPAVLQSSGLYSLSSVVTVPSSSLGTKTYTCNVDHKPSNTKVDKRVESKYGPPCPPCPAPEFLGGPSVFLFPPKPKDTLMISRTPEVTCVVVDVSQEDPEVQFNWYVDGVEVHNAKTKPREEQFNSTYRVVSVLTVLHQDWLNGKEYKCKVSNKGLPSSIEKTISKAKGQPREPQVYTLPPSQEEMTKNQVSLTCLVKGFYPSDIAVEWESNGQPENNYKTTPPVLDSDGSFFLYSRLTVDKSRWQEGNVFSCSVMHEALHNHYTQKSLSLSLGK

SEQ ID NO: 78 - protein, 219 aa, Artificial sequence
  AB613 light chain amino acid sequence
DIVMTQSPDSLAVSLGERATINCKSSQSLLNSRTRKTYLAWYQQKPGESPKLLIYWASTRDSGVPDRFSGSGSGTDFTLTISSLQAEDVAVYYCVQSYTLRTFGGGTKVEIKRTVAAPSVFIFPPSDEQLKSGTASVVCLLNNFYPREAKVQWKVDNALQSGNSQESVTEQDSKDSTYSLSSTLTLSKADYEKHKVYACEVTHQGLSSPVTKSFNRGEC

SEQ ID NO: 79 - DNA, 1338 bp, Artificial sequence
  AB613 heavy chain nucleotide sequence
gaagtgcagctggtgcagtctggcgctgaggtgaagaagcctggctccagcgtcaaggtgagctgcaaggcttctggctacacctttacaagctactatatccactgggtgcgccaggctccaggacagggactggagtggatgggctggatctatcctggcgagggcagcaccaagttcaacgagaagtttaggggccggaccacactgacagccgataagagcaccaatacagcttacatggagctgtcttccctgagatctgaggacaccgccgtgtacttctgcgctcgcgagggctattctctgtattactttgagttttggggtcagggtactacagtgaccgtgagctctgcctctaccaagggcccttccgtgttccctctggccccatgttcccgcagcacctctgagtccacagccgctctgggctgcctggtgaaggactatttccccgagcctgtgaccgtgtcctggaacagcggcgctctgacctccggagtgcacacatttcccgccgtgctgcagtcttccggcctgtacagcctgagctctgtggtgaccgtgccatccagctctctgggcaccaagacatatacctgtaacgtggatcataagccctccaatacaaaggtggacaagcgcgtggagagcaagtacggaccaccatgtcctccatgcccagctcccgagtttctgggcggccctagcgtgttcctgtttccccctaagccaaaggataccctgatgatcagcaggacccctgaggtgacatgcgtggtggtggacgtgtcccaggaggacccagaggtgcagttcaactggtacgtggacggcgtggaggtgcacaatgccaagaccaagcctcgggaggagcagtttaattccacctacagagtggtgagcgtgctgacagtgctgcatcaggactggctgaacggcaaggagtataagtgtaaggtgtccaataagggcctgccatccagcatcgagaagaccatcagcaaggctaagggccagcccagggagcctcaggtgtacacactgccaccctctcaggaggagatgaccaagaaccaggtgtccctgacatgcctggtgaagggcttctatccttccgatatcgccgtggagtgggagagcaatggccagccagagaacaattacaagaccacacctccagtgctggattctgacggctccttctttctgtattcccggctgaccgtggacaagagcagatggcaggagggcaacgtgtttagctgttctgtgatgcatgaggctctgcacaatcattacacacagaagtccctgagcctgtctctgggcaag

SEQ ID NO: 80 - DNA, 657 bp, Artificial sequence
  AB613 light chain nucleotide sequence
gacattgtgatgacacagtctccagactccctggccgtgtccctgggagagagagctaccatcaactgtaagtccagccagtccctgctgaactctaggactagaaagacatacctggcatggtaccagcagaagcccggcgagtctcctaaactgctgatctactgggcctctaccagagattccggagtgccagaccgcttctctggatccggcagcggcacagacttcaccctgacaatctcttccctgcaggccgaggacgtggccgtgtactactgcgtgcagtcttataccctgcgcacatttggcggcggcaccaaggtggagatcaagaggaccgtggctgccccctccgtgttcatctttcccccttccgatgagcagctgaagtccggcacagccagcgtggtgtgcctgctgaacaatttctaccctagagaggctaaggtgcagtggaaggtggacaacgccctgcagagcggcaattctcaggagtccgtgaccgagcaggatagcaaggactctacatattccctgtccagcacactgaccctgagcaaggctgattacgagaagcacaaggtgtatgcctgtgaggtgacccatcagggcctgtcttcccctgtgacaaagtctttcaaccggggcgagtgc

SEQ ID NO: 81 - protein, 452 aa, Artificial sequence
  AB614 heavy chain amino acid sequence
EVQLLESGGGLVQPGGSLKLSCAASGFTFNTYAMNWVRQAPGKGLEWVGRIRSKINNYATYYADSVKDRFTISRDDSKNTAYLQMNNLKTEDTAMYYCVRHDNFYGSTYSWFADWGQGTLVTVSSASTKGPSVFPLAPCSRSTSESTAALGCLVKDYFPEPVTVSWNSGALTSGVHTFPAVLQSSGLYSLSSVVTVPSSSLGTKTYTCNVDHKPSNTKVDKRVESKYGPPCPPCPAPEFLGGPSVFLFPPKPKDTLMISRTPEVTCVVVDVSQEDPEVQFNWYVDGVEVHNAKTKPREEQFNSTYRVVSVLTVLHQDWLNGKEYKCKVSNKGLPSSIEKTISKAKGQPREPQVYTLPPSQEEMTKNQVSLTCLVKGFYPSDIAVEWESNGQPENNYKTTPPVLDSDGSFFLYSRLTVDKSRWQEGNVFSCSVMHEALHNHYTQKSLSLSLGK

SEQ ID NO: 82 - protein, 216 aa, Artificial sequence
  AB614 light chain amino acid sequence
ELVVTQEPSLTVSPGGTVTLTCRSSTGVVTTSNYANWVQEKPDHLFTGLIGATNYRAPGTPARFSGSLLGGKAALTLSGVQPEDEAIYFCVLWYSNHWVFGGGTKLTVLRTVAAPSVFIFPPSDEQLKSGTASVVCLLNNFYPREAKVQWKVDNALQSGNSQESVTEQDSKDSTYSLSSTLTLSKADYEKHKVYACEVTHQGLSSPVTKSFNRGEC

SEQ ID NO: 83 - DNA, 1356 bp, Artificial sequence
  AB614 heavy chain nucleotide sequence
gaggtgcagctgctggagtccggaggaggactggtgcagccaggaggctccctgaagctgagctgtgctgcctctggctttaccttcaacacatatgccatgaattgggtgcggcaggctccaggcaagggactggagtgggtgggcaggatcaggtctaagatcaacaattatgccacctactatgctgattccgtgaaggacaggttcaccatctcccgcgacgatagcaagaacacagcctacctgcagatgaacaatctgaagaccgaggataccgccatgtactactgcgtgagacatgacaacttttacggcagcacatactcctggttcgctgactggggacagggcaccctggtcacagtgagctctgcctctaccaagggcccttccgtgttccctctggccccatgttcccgcagcacctctgagtccacagccgctctgggctgcctggtgaaggactatttccccgagcctgtgaccgtgtcctggaacagcggcgctctgacctccggagtgcacacatttcccgccgtgctgcagtcttccggcctgtacagcctgagctctgtggtgaccgtgccatccagctctctgggcaccaagacatatacctgtaacgtggatcataagccctccaatacaaaggtggacaagcgcgtggagagcaagtacggaccaccatgtcctccatgcccagctcccgagtttctgggcggccctagcgtgttcctgtttccccctaagccaaaggataccctgatgatcagcaggacccctgaggtgacatgcgtggtggtggacgtgtcccaggaggacccagaggtgcagttcaactggtacgtggacggcgtggaggtgcacaatgccaagaccaagcctcgggaggagcagtttaattccacctacagagtggtgagcgtgctgacagtgctgcatcaggactggctgaacggcaaggagtataagtgtaaggtgtccaataagggcctgccatccagcatcgagaagaccatcagcaaggctaagggccagcccagggagcctcaggtgtacacactgccaccctctcaggaggagatgaccaagaaccaggtgtccctgacatgcctggtgaagggcttctatccttccgatatcgccgtggagtgggagagcaatggccagccagagaacaattacaagaccacacctccagtgctggattctgacggctccttctttctgtattcccggctgaccgtggacaagagcagatggcaggagggcaacgtgtttagctgttctgtgatgcatgaggctctgcacaatcattacacacagaagtccctgagcctgtctctgggcaag

SEQ ID NO: 84 - DNA, 648 bp, Artificial sequence
  AB614 light chain nucleotide sequence
gagctggtggtgacccaggagccatctctgacagtgtcccccggcggcacagtgaccctgacatgtagatccagcaccggcgtggtgaccacatccaactacgctaattgggtgcaggagaagccagatcacctgttcacaggactgatcggagctaccaactacagggctcctggaacaccagctcggtttagcggatctctgctgggaggcaaggctgccctgaccctgtccggagtgcagccagaggatgaggccatctacttctgcgtgctgtggtatagcaatcattgggtgttcggaggaggaaccaagctgacagtgctgaggaccgtggctgccccctccgtgttcatctttcccccttccgatgagcagctgaagtccggcacagccagcgtggtgtgcctgctgaacaatttctaccctagagaggctaaggtgcagtggaaggtggacaacgccctgcagagcggcaattctcaggagtccgtgaccgagcaggatagcaaggactctacatattccctgtccagcacactgaccctgagcaaggctgattacgagaagcacaaggtgtatgcctgtgaggtgacccatcagggcctgtcttcccctgtgacaaagtctttcaaccggggcgagtgc

SEQ ID NO: 85 - protein, 8 aa, Artificial sequence
  CDR-H1
GFDFNTYA

SEQ ID NO: 86 - protein, 8 aa, Artificial sequence
  CDR-H1
GFTFDTYA

SEQ ID NO: 87 - protein, 5 aa, Artificial sequence
  CDR-H1
DYAMN

SEQ ID NO: 88 - protein, 8 aa, Artificial sequence
  CDR-H1
GFTFNDYA

SEQ ID NO: 89 - protein, 7 aa, Artificial sequence
  CDR-L2
DTNYRAP

SEQ ID NO: 90 - protein, 3 aa, Artificial sequence
  CDR-L2
DTN

SEQ ID NO: 91 - protein, 7 aa, Artificial sequence
  CDR-L2
ATDYRAP

SEQ ID NO: 92 - protein, 3 aa, Artificial sequence
  CDR-L2
ATD

SEQ ID NO: 93 - protein, 14 aa, Artificial sequence
  CDR-L1
RSSTGVVTTSNHAN

SEQ ID NO: 94 - protein, 9 aa, Artificial sequence
  CDR-L1
TGVVTTSNH

SEQ ID NO: 95 - protein, 7 aa, Artificial sequence
  CDR-L2
ATNHRAP

SEQ ID NO: 96 - protein, 14 aa, Artificial sequence
  CDR-H3
HDNHYGSTYSWFAD

SEQ ID NO: 97 - protein, 16 aa, Artificial sequence
  CDR-H3
VRHDNHYGSTYSWFAD

SEQ ID NO: 98 - protein, 14 aa, Artificial sequence
  CDR-H3
HDNFHGSTYSWFAD

SEQ ID NO: 99 - protein, 16 aa, Artificial sequence
  CDR-H3
VRHDNFHGSTYSWFAD

SEQ ID NO: 100 - protein, 14 aa, Artificial sequence
  CDR-H3
HDNFYGSTHSWFAD

SEQ ID NO: 101 - protein, 16 aa, Artificial sequence
  CDR-H3
VRHDNFYGSTHSWFAD

SEQ ID NO: 102 - protein, 14 aa, Artificial sequence
  CDR-H3
HDNFYGSTYSHFAD

SEQ ID NO: 103 - protein, 16 aa, Artificial sequence
  CDR-H3
VRHDNFYGSTYSHFAD

SEQ ID NO: 104 - protein, 14 aa, Artificial sequence
  CDR-H3
HDNFYGSTYSWHAD

SEQ ID NO: 105 - protein, 16 aa, Artificial sequence
  CDR-H3
VRHDNFYGSTYSWHAD

SEQ ID NO: 106 - protein, 125 aa, Artificial sequence
  AB615 heavy chain variable region
EVQLLESGGGLVQPGGSLKLSCAASGFDFNTYAMNWVRQAPGKGLEWVGRIRSKINNYATYYADSVKDRFTISRDDSKNTAYLQMNNLKTEDTAMYYCVRHDNFYGSTYSWFADWGQGTLVTVSS

SEQ ID NO: 107 - protein, 125 aa, Artificial sequence
  AB616 heavy chain variable region
EVQLLESGGGLVQPGGSLKLSCAASGFTFDTYAMNWVRQAPGKGLEWVGRIRSKINNYATYYADSVKDRFTISRDDSKNTAYLQMNNLKTEDTAMYYCVRHDNFYGSTYSWFADWGQGTLVTVSS

SEQ ID NO: 108 - protein, 125 aa, Artificial sequence
  AB617 heavy chain variable region
EVQLLESGGGLVQPGGSLKLSCAASGFTFNDYAMNWVRQAPGKGLEWVGRIRSKINNYATYYADSVKDRFTISRDDSKNTAYLQMNNLKTEDTAMYYCVRHDNFYGSTYSWFADWGQGTLVTVSS

SEQ ID NO: 109 - protein, 109 aa, Artificial sequence
  AB618 light chain variable region
ELVVTQEPSLTVSPGGTVTLTCRSSTGVVTTSNYANWVQEKPDHLFTGLIGDTNYRAPGTPARFSGSLLGGKAALTLSGVQPEDEAIYFCVLWYSNHWVFGGGTKLTVL

SEQ ID NO: 110 - protein, 109 aa, Artificial sequence
  AB619 light chain variable region
ELVVTQEPSLTVSPGGTVTLTCRSSTGVVTTSNYANWVQEKPDHLFTGLIGATDYRAPGTPARFSGSLLGGKAALTLSGVQPEDEAIYFCVLWYSNHWVFGGGTKLTVL

SEQ ID NO: 111 - protein, 125 aa, Artificial sequence; identical to SEQ ID NO: 107
  AB620 heavy chain variable region

SEQ ID NO: 112 - protein, 109 aa, Artificial sequence; identical to SEQ ID NO: 110
  AB620 light chain variable region

SEQ ID NO: 113 - protein, 109 aa, Artificial sequence
  AB621 light chain variable region
ELVVTQEPSLTVSPGGTVTLTCRSSTGVVTTSNHANWVQEKPDHLFTGLIGATNYRAPGTPARFSGSLLGGKAALTLSGVQPEDEAIYFCVLWYSNHWVFGGGTKLTVL

SEQ ID NO: 114 - protein, 109 aa, Artificial sequence
  AB622 light chain variable region
ELVVTQEPSLTVSPGGTVTLTCRSSTGVVTTSNYANWVQEKPDHLFTGLIGATNHRAPGTPARFSGSLLGGKAALTLSGVQPEDEAIYFCVLWYSNHWVFGGGTKLTVL

SEQ ID NO: 115 - protein, 125 aa, Artificial sequence
  AB623 heavy chain variable region
EVQLLESGGGLVQPGGSLKLSCAASGFTFNTYAMNWVRQAPGKGLEWVGRIRSKINNYATYYADSVKDRFTISRDDSKNTAYLQMNNLKTEDTAMYYCVRHDNHYGSTYSWFADWGQGTLVTVSS

SEQ ID NO: 116 - protein, 125 aa, Artificial sequence
  AB624 heavy chain variable region
EVQLLESGGGLVQPGGSLKLSCAASGFTFNTYAMNWVRQAPGKGLEWVGRIRSKINNYATYYADSVKDRFTISRDDSKNTAYLQMNNLKTEDTAMYYCVRHDNFHGSTYSWFADWGQGTLVTVSS

SEQ ID NO: 117 - protein, 125 aa, Artificial sequence
  AB625 heavy chain variable region
EVQLLESGGGLVQPGGSLKLSCAASGFTFNTYAMNWVRQAPGKGLEWVGRIRSKINNYATYYADSVKDRFTISRDDSKNTAYLQMNNLKTEDTAMYYCVRHDNFYGSTHSWFADWGQGTLVTVSS

SEQ ID NO: 118 - protein, 125 aa, Artificial sequence
  AB626 heavy chain variable region
EVQLLESGGGLVQPGGSLKLSCAASGFTFNTYAMNWVRQAPGKGLEWVGRIRSKINNYATYYADSVKDRFTISRDDSKNTAYLQMNNLKTEDTAMYYCVRHDNFYGSTYSHFADWGQGTLVTVSS

SEQ ID NO: 119 - protein, 125 aa, Artificial sequence
  AB627 heavy chain variable region
EVQLLESGGGLVQPGGSLKLSCAASGFTFNTYAMNWVRQAPGKGLEWVGRIRSKINNYATYYADSVKDRFTISRDDSKNTAYLQMNNLKTEDTAMYYCVRHDNFYGSTYSWHADWGQGTLVTVSS